European Patent Application EP 4 435 097 A1, published September 25, 2024. Title: 具有糖苷水解酶活性的多肽及其制备方法和应用. Applicant: 山东恒鲁生物科技有限公司. The sequence listing filed with the application follows.

SEQUENCE LISTING (40 sequences)

SEQ ID NO: 1 - protein, 722 aa, Bacillus mycoides or Bacillus cereus
MKKKKGRVTLPSEENFLKETKELMERWGADAIRDSDGTKLDDDIKQLDAKIYTTYFVARAHNEFAEKHMDECQQLYLMSLFNTSLTDTLEIDFMKGYFEEQLKPDYVHNPKKYWEVIDRTTGEVVDVNDWEVNEEQNRVLITKAIPWHEYTVSFLVYAIWDPTQMYNHITNNWGDKPHDIPFDVRQPHSNEFMKTYLKQWLTENPDTDVVRFTTFFYHFTLVFNNLGKEKFVDWFGYGASVSVAALDTFQKEKGYRLRPEDIVDQGYYNTAFRIPTPAFLDYIDFVHKFVAEEAKKLVDIVHESGKEAMMFLGDNWIGTEPYGKYFENIGLDAVVGSVGGGATLRMIADIPHVRYTEGRFLPYFFPDTFYEGNNPTIEANENWLTARRALLRNPVDRIGYGGYLSLAYQFPEFISYIEKVTEEFREIHDTIKGVQPYSGLKVAILNSWGKLRTWQTHMVAHALWYKQIYSYLGVLESLSGAAVEVSFISFDDVINDGIPEDIDVIINAGDVGTAFSGGANWINEKLVTTIRAWMYNGGGFIGIGEPTAYQHEGHYFQLANVLGVDKELGFSLSTDKYFINPVENHFISADSTQFDFGEGMKNIYALSEETEIIEYSNGEVHLSSHQFGEGRSVYIAGLPYSEENTRLLMRALYYAAHKEAEFHKYHASNIYCEVHAYPSIQKMAIVNNSMIEQKTVVYDGQGNRKEVTLAPSEIRWEDVSNE

SEQ ID NO: 2 - DNA, 2166 bp, Bacillus mycoides
  source 1..2166: mol_type = other DNA
atgaagaaaaagaaaggccgcgtgaccctgccgagcgaagaaaactttctgaaagaaaccaaagagctgatggaacgctggggcgcggatgcgattcgcgattcagatggcaccaaactggatgatgatattaaacagctggatgcgaaaatttacaccacctattttgtggcgcgtgcccacaacgaatttgcggaaaaacatatggatgaatgccagcagctgtatctgatgagcctgtttaacaccagcctgaccgataccctggaaattgattttatgaaaggctatttcgaggaacagctgaaaccggattatgtgcataacccgaaaaagtattgggaggtgattgatcgcaccaccggcgaagtggtggatgtgaacgattgggaagtgaacgaagaacagaaccgcgtgctgattaccaaagcgattccgtggcatgaatataccgtgagctttctggtgtatgcgatttgggatccgacccagatgtataaccatattaccaacaactggggcgataaaccgcatgatattccgtttgatgtgcgccagccgcatagcaacgaatttatgaaaacctatctgaaacagtggctgaccgaaaacccggataccgatgtggtgcgctttaccacctttttctatcattttaccctggtgtttaacaacctgggcaaagaaaaatttgtggactggtttggctatggcgcgagcgtgagcgtggcggcattagatacctttcagaaagaaaaaggctatcgcctgcgcccggaagatattgtggatcagggctattataacaccgcgtttcgcattccgaccccggcgtttctggattatattgattttgtgcataagttcgtggcggaggaggcgaaaaagctggtggatattgtgcatgaaagcggcaaagaagcgatgatgtttctgggcgataactggattggcaccgaaccgtatggcaaatattttgaaaacattggcctggacgcggtggtgggcagcgtgggtggtggtgcgactttacgtatgattgcggatattccgcatgtgcgctataccgaaggccgctttctgccgtatttctttccggataccttttatgaaggcaacaacccgaccattgaagcgaacgaaaactggctgaccgcccgccgcgcgttattacgcaatccggttgatcgtattggctatggcggctatctgagcctggcgtatcagtttccggaatttattagctatattgagaaagtgaccgaggagttccgcgaaattcatgataccattaaaggcgtgcagccgtatagcggcctgaaagtggcgattctgaacagctggggcaaactgcgcacctggcagacccatatggtggcgcatgcgctgtggtataaacagatttatagctatctgggcgtgctggaaagcctgagcggcgcggcggttgaagttagctttattagctttgatgatgtgattaacgacggcattccggaagatattgatgtgattattaacgcgggcgatgtgggcaccgcgtttagcggtggtgcaaattggattaacgaaaaactggtgacgaccattcgcgcgtggatgtataacggcggcggctttattggcattggcgaaccgaccgcgtatcagcatgaaggccattattttcagctggcgaacgtgctgggcgtggataaagaactgggctttagcctgagcaccgataaatattttattaacccggtggaaaaccacttcatcagcgcggatagcacccagtttgattttggcgaaggcatgaaaaacatttatgcgctgagcgaagaaaccgaaattattgaatatagcaacggcgaagtgcatctgagcagccatcagtttggcgaaggccgcagcgtgtatattgcgggcttaccgtatagcgaagaaaacacccgcctgctgatgcgagcgctgtattatgcggcgcataaagaagcggaatttcataaatatcacgcgagcaacatttactgcgaagtgcatgcgtatccgagcattcagaaaatggcgattgtgaacaacagcatgattgaacagaaaaccgtggtgtatgatggccagggcaaccgcaaagaagtgaccctggcgccgagcgaaattcgctgggaagatgtgagcaacgaa

SEQ ID NO: 3 - DNA, 48 bp, synthetic construct
  source 1..48: mol_type = other DNA
atcggatccgaattcaaaaagaaaaaaggccgtgttactttaccgagt

SEQ ID NO: 4 - DNA, 33 bp, synthetic construct
  source 1..33: mol_type = other DNA
tgcggccgcaagcttgccttcatttgaaacatc

SEQ ID NO: 5 - DNA, 48 bp, synthetic construct
  source 1..48: mol_type = other DNA
gataagcttatgaaaaagaaaaaaggccgtgttactttaccgagtgaa

SEQ ID NO: 6 - DNA, 32 bp, synthetic construct
  source 1..32: mol_type = other DNA
caggaattcgccttcatttgaaacatcctccc

SEQ ID NO: 7 - DNA, 35 bp, synthetic construct
  source 1..35: mol_type = other DNA
gaagcttacgtaatgacttctactggtagattcac

SEQ ID NO: 8 - DNA, 53 bp, synthetic construct
  source 1..53: mol_type = other DNA
tcaaggccttaattaagcggccgcttagtggtgatggtggtgatgcaaatttc

SEQ ID NO: 9 - DNA, 26 bp, synthetic construct
  source 1..26: mol_type = other DNA
gacgcagatcgggaacactgaaaaat

SEQ ID NO: 10 - DNA, 35 bp, synthetic construct
  source 1..35: mol_type = other DNA
actttgatttctctggattcggaatggtttgaacg

SEQ ID NO: 11 - DNA, 53 bp, synthetic construct
  source 1..53: mol_type = other DNA
agctagaagagctagatctcctaggatgacttctactggtagattcactttgc

SEQ ID NO: 12 - DNA, 49 bp, synthetic construct
  source 1..49: mol_type = other DNA
tcaaggccttaattaagcggccgcttagtggtgatggtggtgatgcaaa

SEQ ID NO: 13 - DNA, 34 bp, synthetic construct
  source 1..34: mol_type = other DNA
ccgcggggatcgactcataaaatagtaaccttct

SEQ ID NO: 14 - DNA, 35 bp, synthetic construct
  source 1..35: mol_type = other DNA
gccgcggaaatttaggaattttaaacttgggcttg

SEQ ID NO: 15 - DNA, 44 bp, synthetic construct
  source 1..44: mol_type = other DNA
caattacaagagaacttctactggtagattcactttgccatctg

SEQ ID NO: 16 - DNA, 42 bp, synthetic construct
  source 1..42: mol_type = other DNA
atggtggtgatgcaaatttctccaagcaatagcagattgatc

SEQ ID NO: 17 - DNA, 29 bp, synthetic construct
  source 1..29: mol_type = other DNA
caaaccgaaatggggcgttgttaccccag

SEQ ID NO: 18 - DNA, 40 bp, synthetic construct
  source 1..40: mol_type = other DNA
accagtagaagttctcttgtaattgataactgaagcactg

SEQ ID NO: 19 - DNA, 44 bp, synthetic construct; identical to SEQ ID NO: 15
  source 1..44: mol_type = other DNA

SEQ ID NO: 20 - DNA, 30 bp, synthetic construct
  source 1..30: mol_type = other DNA
cctccatgtcccggtagaggtgtggtcaat

SEQ ID NO: 21 - DNA, 30 bp, synthetic construct
  source 1..30: mol_type = other DNA
cctctaccgggacatggaggcccagaatac

SEQ ID NO: 22 - DNA, 32 bp, synthetic construct
  source 1..32: mol_type = other DNA
aagcagatcagacagtatagcgaccagcattc

SEQ ID NO: 23 - DNA, 37 bp, synthetic construct
  source 1..37: mol_type = other DNA
tcgctatactgtctgatctgcttactttactaacgac

SEQ ID NO: 24 - DNA, 32 bp, synthetic construct
  source 1..32: mol_type = other DNA
tcgtggcagcaattcatgatcgtaacgtggta

SEQ ID NO: 25 - DNA, 30 bp, synthetic construct
  source 1..30: mol_type = other DNA
acaacctgggcaaannnaaatttgtggact

SEQ ID NO: 26 - DNA, 30 bp, synthetic construct
  source 1..30: mol_type = other DNA
agtccacaaatttnnntttgcccaggttgt

SEQ ID NO: 27 - DNA, 35 bp, synthetic construct
  source 1..35: mol_type = other DNA
caaagaaaaatttgtgnnntggtttggctaggcgc

SEQ ID NO: 28 - DNA, 35 bp, synthetic construct
  source 1..35: mol_type = other DNA
gcgcctagccaaaccannncacaaatttttctttg

SEQ ID NO: 29 - DNA, 40 bp, synthetic construct
  source 1..40: mol_type = other DNA
atcagggctattataacaccnnntttcgcattccgacccc

SEQ ID NO: 30 - DNA, 40 bp, synthetic construct
  source 1..40: mol_type = other DNA
ggggtcggaatgcgaaannnggtgttataatagccctgat

SEQ ID NO: 31 - DNA, 35 bp, synthetic construct
  source 1..35: mol_type = other DNA
tggcaccgaaccgtatnnnaaatattttgaaaaca

SEQ ID NO: 32 - DNA, 35 bp, synthetic construct
  source 1..35: mol_type = other DNA
tgttttcaaaatatttnnnatacggttcggtgcca

SEQ ID NO: 33 - DNA, 32 bp, synthetic construct
  source 1..32: mol_type = other DNA
tggtgggcagcgtgnnnggtggtgcgacttta

SEQ ID NO: 34 - DNA, 32 bp, synthetic construct
  source 1..32: mol_type = other DNA
taaagtcgcaccaccnnncacgctgcccacca

SEQ ID NO: 35 - DNA, 36 bp, synthetic construct
  source 1..36: mol_type = other DNA
cgtgggtggtggtgcgnnnttacgtatgattgcgga

SEQ ID NO: 36 - DNA, 36 bp, synthetic construct
  source 1..36: mol_type = other DNA
tccgcaatcatacgtaannncgcaccaccacccacg

SEQ ID NO: 37 - DNA, 35 bp, synthetic construct
  source 1..35: mol_type = other DNA
tggcagacccatatgnnngcgatgcgctgtggtat

SEQ ID NO: 38 - DNA, 35 bp, synthetic construct
  source 1..35: mol_type = other DNA
ataccacagcgcatcgcnnncatatgggtctgcca

SEQ ID NO: 39 - DNA, 37 bp, synthetic construct
  source 1..37: mol_type = other DNA
cgcagacccatatggtgnnncatgcgctgtggtataa

SEQ ID NO: 40 - DNA, 37 bp, synthetic construct
  source 1..37: mol_type = other DNA
ttataccacagcgcatgnnncaccatatgggtctgcg